European Patent Specification EP 3 341 485 B1, published November 26, 2025. Title: Enhanced Production of Immunglobulin. Applicant: Trianni, Inc. Application Submitted Herewith. The sequence listing filed with the application follows.

SEQUENCE LISTING (5 sequences)

SEQ ID NO: 1 - DNA, 1182 bp, Mus musculus
gccaaaacgacacccccatctgtctatccactggcccctggatctgctgcccaaactaactccatggtgaccctgggatgcctggtcaagggctatttccctgagccagtgacagtgacctggaactctggatccctgtccagcggtgtgcacaccttcccagctgtcctgcagtctgacctctacactctgagcagctcagtgactgtcccctccagcacctggcccagccagaccgtcacctgcaacgttgcccacccggccagcagcaccaaggtggacaagaaaattgtgcccagggattgtggttgtaagccttgcatatgtacagtcccagaagtatcatctgtcttcatcttccccccaaagcccaaggatgtgctcaccattactctgactcctaaggtcacgtgtgttgtggtagacatcagcaaggatgatcccgaggtccagttcagctggtttgtagatgatgtggaggtgcacacagctcagacgaaaccccgggaggagcagatcaacagcactttccgttcagtcagtgaacttcccatcatgcaccaggactggctcaatggcaaggagttcaaatgcagggtcaacagtgcagctttccctgcccccatcgagaaaaccatctccaaaaccaaaggcagaccgaaggctccacaggtgtacaccattccacctcccaagaaaaagatggccaaggataaagtcagtctgacctgcatgataacaaacttcttccctgaagacattactgtggagtggcagtggaatgggcagccagcggagaactacaagaacactcagcccatcatgaagacagatggctcttacttcgtctacagcaagctcaatgtgcagaagagcaactgggaggcaggaaatactttcacctgctctgtgttacatgagggcctgcacaaccaccatactgagaagagcctctcccactctcctgggctgcaactggacgagacctgtgctgaggcccaggacggggagctggacgggctctggacgaccatcaccatcttcatcagcctcttcctgctcagtgtgtgctacagcgctgctgtcacactcttcaaggtaaagtggatcttctcctcggtggtggagctgaagcagacactggttcctgaatacaagaacatgattgggcaagcaccctag

SEQ ID NO: 2 - DNA, 1182 bp, Mus musculus
gccaaaacgacacccccatctgtctatccactggcccctggatctgctgcccaaactaactccatggtgaccctgggatgcctggtcaagggctatttccctgagccagtgacagtgacctggaactctggatccctgtccagcggtgtgcacaccttcccagctgtcctgcagtctgacctctacactctgagcagctcagtgactgtcccctccagcacctggcccagccagaccgtcacctgcaacgttgcccacccggccagcagcaccaaggtggacaagaaaattgtgcccagggattgtggttgtaagccttgcatatgtacagtcccagaagtatcatctgtcttcatcttccccccaaagcccaaggatgtgctcaccattactctgactcctaaggtcacgtgtgttgtggtagacatcagcaaggatgatcccgaggtccagttcagctggtttgtagatgatgtggaggtgcacacagctcagacgaaaccccgggaggagcagatcaacagcactttccgttcagtcagtgaacttcccatcatgcaccaggactggctcaatggcaaggagttcaaatgcagggtcaacagtgcagctttccctgcccccatcgagaaaaccatctccaaaaccaaaggcagaccgaaggctccacaggtgtacaccattccacctcccaaggagcagatggccaaggataaagtcagtctgacctgcatgatagataacttcttccctgaagacattactgtggagtggcagtggaatgggcagccagcggagaactacgataacactcagcccatcatggacacagatggctcttacttcgtctacagcgatctcaatgtgcagaagagcaactgggaggcaggaaatactttcacctgctctgtgttacatgagggcctgcacaaccaccatactgagaagagcctctcccactctcctgggctgcaactggacgagacctgtgctgaggcccaggacggggagctggacgggctctggacgaccatcaccatcttcatcagcctcttcctgctcagtgtgtgctacagcgctgctgtcacactcttcaaggtaaagtggatcttctcctcggtggtggagctgaagcagacactggttcctgaatacaagaacatgattgggcaagcaccctag

SEQ ID NO: 3 - DNA, 1182 bp, Mus musculus
gccaaaacgacacccccatctgtctatccactggcccctggatctgctgcccaaactaactccatggtgaccctgggatgcctggtcaagggctatttccctgagccagtgacagtgacctggaactctggatccctgtccagcggtgtgcacaccttcccagctgtcctgcagtctgacctctacactctgagcagctcagtgactgtcccctccagcacctggcccagccagaccgtcacctgcaacgttgcccacccggccagcagcaccaaggtggacaagaaaattgtgcccagggattgtggttgtaagccttgcatatgtacagtcccagaagtatcatctgtcttcatcttccccccaaagcccaaggatgtgctcaccattactctgactcctaaggtcacgtgtgttgtggtagacatcagcaaggatgatcccgaggtccagttcagctggtttgtagatgatgtggaggtgcacacagctcagacgaaaccccgggaggagcagatcaacagcactttccgttcagtcagtgaacttcccatcatgcaccaggactggctcaatggcaaggagttcaaatgcagggtcaacagtgcagctttccctgcccccatcgagaaaaccatctccaaaaccaaaggcagaccgaaggctccacaggtgtacaccattccacctcccaaggagcagatggccaaggataaagtcagtctgacctgcatgataacaaacttcttccctgaagacattactgtggagtggcagtggaatgggcagccagcggagaactacaagaacactcagcccatcatggacacagatggctcttacttcgtctacagcaagctcaatgtgcagaagagcaactgggaggcaggaaatactttcacctgctctgtgttacatgagggcctgcacaaccaccatactgagaagagcctctcccactctcctgggctgcaactggacgagacctgtgctgaggcccaggacggggagctggacgggctctggacgaccatcaccatcttcatcagcctcttcctgctcagtgtgtgctacagcgctgctgtcacactcttcaaggtaaagtggatcttctcctcggtggtggagctgaagcagacactggttcctgaatacaagaacatgattgggcaagcaccctag

SEQ ID NO: 4 - DNA, 627 bp, Artificial Sequence
  Fusion of splice acceptor, mus musculus Itbg exon 15 with stop codon, mus musculus Itgb7 intron, mus musculus Itgb7 exon with stop codon untranslated region, and polyadenylation sequence
cagagggagtggatcacacccgtgccatcatactgggctgcacagggggcatcgtggcagtgggactagggctggttctggcttactgactctctgtggaaatctacgaccgacgggagtacaggcgctttgagaaggagcagcagcaactcaactggaagcaggtgaggccagcgactgctgccacaggctgggctttcctggtgacgtctcttaactttctgtatccctaacacataaccagctctaaagcttccccgtgcaagtccctccctcggcataaccaggcctcggagatctggcctcgtggggcaggtagtggggagagcctgatagttttccttactgtgtgcaatgttttcccacaggacaacaatcctctctacaaaagtgcgatcacaaccactgtcaacccccgcttccaagggacaaacggtcggtcgccatccctctctctgaccagggaagcagactgacttaggattcttgtcttggaggacagtggagatagaagggcagggcagcgtctgtcaggcaaagatgctgccaccgctgagatttttcagagtgaccttcagagggcagcagccattcccaccacacgaagggctggtccttccataataa

SEQ ID NO: 5 - DNA, 757 bp, Artificial Sequence
  Fusion construct of splice acceptor, linker, PTV-1-2A peptide, mus musculus Bcl2 open reading frame, mus musculus 3' untranslated region, and polyadenylation signal
cagggatccggagccacgaacttctctctgttaaagcaagcaggagacgtggaagaaaaccccggtcctatggcgcaagccgggagaacagggtatgataaccgggagatcgtgatgaagtacatacattataagctgtcacagaggggctacgagtgggatgctggagatgcggacgcggcgcccctgggggctgcccccacccctggcatcttctccttccagcctgagagcaacccaatgcccgctgtgcaccgggacatggctgccaggacgtctcctctcaggcccctcgttgccaccgctgggcctgcgctcagccctgtgccacctgtggtccatctgaccctccgccgggctggggatgacttctctcgtcgctaccgtcgtgacttcgcagagatgtccagtcagctgcacctgacgcccttcaccgcgaggggacgctttgccacggtggtggaggaactcttcagggatggggtgaactgggggaggattgtggccttctttgagttcggtggggtcatgtgtgtggagagcgtcaacagggagatgtcacccctggtggacaacatcgccctgtggatgactgagtacctgaaccggcatctgcacacctggatccaggataacggaggctgggtaggtgcatgtctggttgaatgagtctgggctttgatctcaaggccaagatgcgcaggttggggtgtgagtggattctgggtcaaaatgggccattgagcagatgaaataa